European Patent Application EP 4 144 832 A1, published March 8, 2023. Title: NOVEL LACTOBACILLUS PLANTARUM, LACTIC ACID BACTERIA COMPOSITION AND USE THEREOF FOR CURING OR PREVENTING HEAVY METAL RELATED DISEASES. Applicant: Native Biomedicals Ltd. The sequence listing filed with the application follows.

SEQUENCE LISTING (2 sequences)

SEQ ID NO: 1 - DNA, 1506 bp, Lactobacillus plantarum
gacgaacgctggcggcgtgcctaatacatgcaagtcgaacgaactctggtattgattggtgcttgcatcatgatttacatttgagtgagtggcgaactggtgagtaacacgtgggaaacctgcccagaagcgggggataacacctggaaacagatgctaataccgcataayaacttggaccgcatggtccgagyttgaaagatggcttcggctatcacttttggatggtcccgcggcgtattagctagatggtggggtaacggctcaccatggcaatgatacgtagccgacctgagagggtaatcggccacattgggactgagacacggcccaaactcctacgggaggcagcagtagggaatcttccacaatggacgaaagtctgatggagcaacgccgcgtgagtgaagaagggtttcggctcgtaaaactctgttgttaaagaagaacatatctgagagtaactgttcaggtattgacggtatttaaccagaaagccacggctaactacgtgccagcagccgcggtaatacgtaggtggcaagcgttgtccggatttattgggcgtaaagcgagcgcaggcggttttttaagtctgatgtgaaagccttcggctcaaccgaagaagtgcatcggaaactgggaaacttgagtgcagaagaggacagtggaactccatgtgtagcggtgaaatgcgtagatatatggaagaacaccagtggcgaaggcggctgtctggtctgtaactgacgctgaggctcgaaagtatgggtagcaaacaggattagataccctggtagtccataccgtaaacgatgaatgctaagtgttggagggtttccgcccttcagtgctgcagctaacgcattaagcattccgcctggggagtacggccgcaaggctgaaactcaaaggaattgacgggggcccgcacaagcggtggagcatgtggtttaattcgaagctacgcgaagaaccttaccaggtcttgacatactatgcaaatctaagagattagacgttcccttcggggacatggatacaggtggtgcatggttgtcgtcagctcgtgtcgtgagatgttgggttaagtcccgcaacgagcgcaacccttattatcagttgccagcattaagttgggcactctggtgagctgccggtgacaaaccggaggaaggtggggatgacgtcaaatcatcatgccccttatgacctgggctacacacgtgctacaacgagttgcgaactcgcgagagtaagctaatctcttaaagccattctcagttcggattgtaggctgcaactcgcctacatgaagtcggaatcgctagtaatcgcggatcagcatgccgcggtgaatacgttcccgggccttgtacacaccgcccgtcacaccatgagagtttgtaacacccaaagtcggtggggtaaccttttaggaaccagccgcctaaggtgggacagatgattagggtgaagtcgtaacaaggtagccgtaggagaacc

SEQ ID NO: 2 - DNA, 1516 bp, Lactobacillus delbrueckii
gacgaacgctggcggcgtgcctaatacatgcaagtcgagcgagctgaattcaaagatycyttcgggrtgatttgttggaygctagcggcggatgggtgagtaacacgtgggcaatctgccctaaagactgggataccacttggaaacaggtgctaataccggataacaacatgaatcgcatgattcaagtttgaaaggcggcgcaagctgtcactttaggatgagcccgcggcgcattagctagttggtggggtaaaggcctaccaaggcaatgatgcgtagccgagttgagagactgatcggccacattgggactgagacacggcccaaactcctacgggaggcagcagtagggaatcttccacaatggacgcaagtctgatggagcaacgccgcgtgagtgaagaaggtcttcggatcgtaaagctctgttgttggtgaagaaggatagaggcagtaactggtctttatttgacggtaatcaaccagaaagtcacggctaactacgtgccagcagccgcggtaatacgtaggtggcaagcgttgtccggatttattgggcgtaaagcgagcgcaggcggaatgataagtctgatgtgaaagcccacggctcaaccgtggaactgcatcggaaactgtcattcttgagtgcagaagaggagagtggaactccatgtgtagcggtggaatgcgtagatatatggaagaacaccagtggcgaaggcggctctctggtctgcaactgacgctgaggctcgaaagcatgggtagcgaacaggattagataccctggtagtccatgccgtaaacgatgagcgctaggtgttggggactttccggtyctcagtgccgcagcaaacgcrttaagcgctccgcctggggagtacgaccgcaaggttgaaactcaaaggaattgacgggggcccgcacaagcggtggagcatgtggtttaattcgaagcaacgcgaagaaccttaccaggtcttgacatcctgcgctacacctagagataggtggttcccttcggggacgcagagacaggtggtgcatggctgtcgtcagctggtgtcgtgagatgttgggttaagtcccgcaacgagcgcaacccttgtctttagttgccatcattaagttgggcactctaragagactgccggtgacaaaccggaggaaggtggggatgacgtcaagtcatcatgccccttatgacctgggctacacacgtgctacaatgggcagtacaacgagaagcgaacccgcgagggtaagcggatctcttaaagctgctctcagttcggactgcaggctgcaactcgcctgcacgaagctggaatcgctagtaatcgcggatcagcacgccgcggtgaatacgttcccgggccttgtacacaccgcccgtcacaccatggaagtctgcaatgcccaaagtcggtgrgataacctttataggagtcagccgcctaaggcagggcagatgactggggtgaagtcgtaacaaggtagccgtaggagaacc